European Patent Specification EP 3 393 474 B1, published July 19, 2023. Title: METHOD OF TREATING HETEROTOPIC OSSIFICATION. Applicant: Levi, et al. The sequence listing filed with the application follows.

SEQUENCE LISTING (6 sequences)

SEQ ID NO: 1 - DNA, 22 bp, Mus musculus
  misc_feature: Hif1 alpha- forward primer
gtcccagctacgaagttacagc

SEQ ID NO: 2 - DNA, 22 bp, Mus musculus
  misc_feature: Hif1 alpha- reverse primer
cagtgcaggatacacaaggttt

SEQ ID NO: 3 - DNA, 20 bp, Mus musculus
  misc_feature: Sox9- forward primer
agtacccgcatctgcacaac

SEQ ID NO: 4 - DNA, 20 bp, Mus musculus
  misc_feature: Sox9- reverse primer
acgaagggtctcttctcgct

SEQ ID NO: 5 - DNA, 20 bp, Mus musculus
  misc_feature: Acan- forward primer
actgcgacatctggagtgac

SEQ ID NO: 6 - DNA, 20 bp, Mus musculus
  misc_feature: Acan- reverse primer
ctgtccactgccaaagagaa